European Patent Specification EP 4 086 348 B1, published April 1, 2026. Title: METHODS AND COMPOSITIONS FOR COMBINATIONS OF MUTATIONS ASSOCIATED WITH HERBICIDE RESISTANCE/TOLERANCE IN RICE. Applicant: RICETEC, INC. The sequence listing filed with the application follows.

SEQUENCE LISTING (65 sequences)

SEQ ID NO: 1 - DNA, 2501 bp, Oryza sativa
cctgttctgctaggaataatagaactacatactgctatgattttccactggtgagttgactgctcccttatattcaatgcattaccatagcaaattcatattcgttcatgttgtcaaaataagccgatgaaaattcaaaactgtaggcatttgaaactgcagtgaggaagtcatggtcctctagtacctctggtgcttctaaaggtgttgaaaatgcccaatgttatgttaaagctacagagttggtatttgcggacaaacatgggtcatggggcactcctttagttcaaatggaccggcctgctgggctcaatgacattggtatggtagcttggaccttgaagatgtccactcctgaatttcctagtggtagggagattattgttgttgcaaatgatattacgttcagagctggatcatttggcccaagggaagatgcattttttgaagctgttaccaacctagcctgtgagaagaaacttcctcttatttatttggcagcaaattctggtgctcgaattggcatagcagatgaagtgaaatcttgcttccgtgttgggtggtctgatgatggcagccctgaacgtgggtttcagtacatttatctaagcgaagaagactatgctcgtattggcacttctgtcatagcacataagatgcagctagacagtggtgaaattaggtgggttattgattctgttgtgggcaaggaagatggacttggtgtggagaatatacatggaagtgctgctattgccagtgcttattctagggcatataaggagacatttacacttacatttgtgactggaagaactgttggaataggagcttatcttgctcgacttggcatccggtgcatacagcgtcttgaccagcctattattcttacaggctattctgcactgaacaagcttcttgggcgggaagtgtacagctcccacatgcagttgggtggtcccaaaatcatggcaactaatggtgttgtccatcttactgtttcagatgaccttgaaggcgtttctaatatattgaggtggctcagttatgttcctgcctacattggtggaccacttccagtaacaacaccgttggacccaccggacagacctgttgcatacattcctgagaactcgtgtgatcctcgagcggctatccgtggtgttgatgacagccaagggaaatggttaggtggtatgtttgataaagacagctttgtggaaacatttgaaggttgggctaagacagtggttactggcagagcaaagcttggtggaattccagtgggtgtgatagctgtggagactcagaccatgatgcaaactatccctgctgaccctggtcagcttgattcccgtgagcaatctgttcctcgtgctggacaagtgtggtttccagattctgcaaccaagactgcgcaggcattgctggacttcaaccgtgaaggattacctctgttcatcctcgctaactggagaggcttctctggtggacaaagagatctttttgaaggaattcttcaggctggctcgactattgttgagaaccttaggacatacaatcagcctgcctttgtctacattcccatggctgcagagctacgaggaggggcttgggttgtggttgatagcaagataaacccagaccgcattgagtgctatgctgagaggactgcaaaaggcaatgttctggaaccgcaagggttaattgagatcaagttcaggtcagaggaactccaggattgcatgagtcggcttgacccaacattaattgatctgaaagcaaaactcgaagtagcaaataaaaatggaagtgctgacacaaaatcgcttcaagaaaatatagaagctcgaacaaaacagttgatgcctctatatactcagattgcgatacggtttgctgaattgcatgatacatccctcagaatggctgcgaaaggtgtgattaagaaagttgtggactgggaagaatcacgatctttcttctataagagattacggaggaggatctctgaggatgttcttgcaaaagaaattagagctgtagcaggtgagcagttttcccaccaaccagcaatcgagctgatcaagaaatggtattcagcttcacatgcagctgaatgggatgatgacgatgcttttgttgcttggatggataaccctgaaaactacaaggattatattcaatatcttaaggctcaaagagtatcccaatccctctcaagtctttcagattccagctcagatttgcaagccctgccacagggtctttccatgttactagataaggtaattagcttactgatgcttatataaattctttttcattacatatggctggagaactatctaatcaaataatgattataattccaatcgttctttttatgccattatgatcttctgaaatttccttctttggacacttattcagatggatccctctagaagagctcaacttgttgaagaaatcaggaaggtccttggttgaatcatatgatg

SEQ ID NO: 2 - DNA, 2501 bp, Oryza sativa; identical to SEQ ID NO: 1

SEQ ID NO: 3 - DNA, 2501 bp, Oryza sativa
cctgttctgctaggaataatagaactacatactgctatgattttccactggtgagttgactgctcccttatattcaatgcattaccatagcaaattcatattcgttcatgttgtcaaaataagccgatgaaaattcaaaactgtaggcatttgaaactgcagtgaggaagtcatggtcctctagtacctctggtgcttctaaaggtgttgaaaatgcccaatgttatgttaaagctacagagttggtatttgcggacaaacatgggtcatggggcactcctttagttcaaatggaccggcctgctgggctcaatgacattggtatggtagcttggaccttgaagatgtccactcctgaatttcctagtggtagggagattattgttgttgcaaatgatattacgttcagagctggatcatttggcccaagggaagatgcattttttgaagctgttaccaacctagcctgtgagaagaaacttcctcttatttatttggcagcaaattctggtgctcgaattggcatagcagatgaagtgaaatcttgcttccgtgttgggtggtctgatgatggcagccctgaacgtgggtttcagtacatttatctaagcgaagaagactatgctcgtattggcacttctgtcatagcacataagatgcagctagacagtggtgaaattaggtgggttattgattctgttgtgggcaaggaagatggacttggtgtggagaatatacatggaagtgctgctattgccagtgcttattctagggcatataaggagacatttacacttacatttgtgactggaagaactgttggaataggagcttatcttgctcgacttggcatccggtgcatacagcgtcttgaccagcctattattcttacaggctattctgcactgaacaagcttcttgggcgggaagtgtacagctcccacatgcagttgggtggtcccaaaatcatggcaactaatggtgttgtccatcttactgtttcagatgaccttgaaggcgtttctaatatattgaggtggctcagttatgttcctgcctacattggtggaccacttccagtaacaacaccgttggacccaccggacagacctgttgcatacattcctgagaactcgtgtgatcctcgagcggctatccgtggtgttgatgacagccaagggaaatggttaggtggtatgtttgataaagacagctttgtggaaacatttgaaggttgggctaagacagtggttactggcagagcaaagcttggtggaattccagtgggtgtgatagctgtggagactcagaccatgatgcaaactatccctgctgaccctggtcagcttgattcccgtgagcaatctgttcctcgtgctggacaagtgtggtttccagattctgcaaccaagactgcgcaggcattgctggacttcaaccgtgaaggattacctctgttcatcctcgctaactggagaggcttctctggtggacaaagagatctttttgaaggaattcttcaggctggctcgactattgttgagaaccttaggacatacaatcagcctgcctttgtctacattcccatggctgcagagctacgaggaggggcttgggttgtggttgatagcaagataaacccagaccgcattgagtgctatgctgagaggactgcaaaaagcaatgttctggaaccgcaagggttaattgagatcaagttcaggtcagaggaactccaggattgcatgagtcggcttgacccaacattaattgatctgaaagcaaaactcgaagtagcaaataaaaatggaagtgctgacacaaaatcgcttcaagaaaatatagaagctcgaacaaaacagttgatgcctctatatactcagattgcgatacggtttgctgaattgcatgatacatccctcagaatggctgcgaaaggtgtgattaagaaagttgtggactgggaagaatcacgatctttcttctataagagattacggaggaggatctctgaggatgttcttgcaaaagaaattagagctgtagcaggtgagcagttttcccaccaaccagcaatcgagctgatcaagaaatggtattcagcttcacatgcagctgaatgggatgatgacgatgcttttgttgcttggatggataaccctgaaaactacaaggattatattcaatatcttaaggctcaaagagtatcccaatccctctcaagtctttcagattccagctcagatttgcaagccctgccacagggtctttccatgttactagataaggtaattagcttactgatgcttatataaattctttttcattacatatggctggagaactatctaatcaaataatgattataattccaatcgttctttttatgccattatgatcttctgaaatttccttctttggacacttattcagatggatccctctagaagagctcaacttgttgaagaaatcaggaaggtccttggttgaatcatatgatg

SEQ ID NO: 4 - protein, 674 aa, Oryza sativa
MDRPAGLNDIGMVAWTLKMSTPEFPSGREIIVVANDITFRAGSFGPREDAFFEAVTNLACEKKLPLIYLAANSGARIGIADEVKSCFRVGWSDDGSPERGFQYIYLSEEDYARIGTSVIAHKMQLDSGEIRWVIDSVVGKEDGLGVENIHGSAAIASAYSRAYKETFTLTFVTGRTVGIGAYLARLGIRCIQRLDQPIILTGYSALNKLLGREVYSSHMQLGGPKIMATNGVVHLTVSDDLEGVSNILRWLSYVPAYIGGPLPVTTPLDPPDRPVAYIPENSCDPRAAIRGVDDSQGKWLGGMFDKDSFVETFEGWAKTVVTGRAKLGGIPVGVIAVETQTMMQTIPADPGQLDSREQSVPRAGQVWFPDSATKTAQALLDFNREGLPLFILANWRGFSGGQRDLFEGILQAGSTIVENLRTYNQPAFVYIPMAAELRGGAWVVVDSKINPDRIECYAERTAKGNVLEPQGLIEIKFRSEELQDCMSRLDPTLIDLKAKLEVANKNGSADTKSLQENIEARTKQLMPLYTQIAIRFAELHDTSLRMAAKGVIKKVVDWEESRSFFYKRLRRRISEDVLAKEIRAVAGEQFSHQPAIELIKKWYSASHAAEWDDDDAFVAWMDNPENYKDYIQYLKAQRVSQSLSSLSDSSSDLQALPQGLSMLLDKVISLLMLI

SEQ ID NO: 5 - protein, 674 aa, Oryza sativa; identical to SEQ ID NO: 4

SEQ ID NO: 6 - protein, 674 aa, Oryza sativa
MDRPAGLNDIGMVAWTLKMSTPEFPSGREIIVVANDITFRAGSFGPREDAFFEAVTNLACEKKLPLIYLAANSGARIGIADEVKSCFRVGWSDDGSPERGFQYIYLSEEDYARIGTSVIAHKMQLDSGEIRWVIDSVVGKEDGLGVENIHGSAAIASAYSRAYKETFTLTFVTGRTVGIGAYLARLGIRCIQRLDQPIILTGYSALNKLLGREVYSSHMQLGGPKIMATNGVVHLTVSDDLEGVSNILRWLSYVPAYIGGPLPVTTPLDPPDRPVAYIPENSCDPRAAIRGVDDSQGKWLGGMFDKDSFVETFEGWAKTVVTGRAKLGGIPVGVIAVETQTMMQTIPADPGQLDSREQSVPRAGQVWFPDSATKTAQALLDFNREGLPLFILANWRGFSGGQRDLFEGILQAGSTIVENLRTYNQPAFVYIPMAAELRGGAWVVVDSKINPDRIECYAERTAKSNVLEPQGLIEIKFRSEELQDCMSRLDPTLIDLKAKLEVANKNGSADTKSLQENIEARTKQLMPLYTQIAIRFAELHDTSLRMAAKGVIKKVVDWEESRSFFYKRLRRRISEDVLAKEIRAVAGEQFSHQPAIELIKKWYSASHAAEWDDDDAFVAWMDNPENYKDYIQYLKAQRVSQSLSSLSDSSSDLQALPQGLSMLLDKVISLLMLI

SEQ ID NO: 7 - DNA, 201 bp, Oryza sativa
ataaagatgaggtgtttgatgaattaaaggccgcagggttgaagaggccatgtagctttacagatatttccagtgaaaatgctttgcttcttgaatttgakacagcaactgatgcagctgctgcgaaagcccatattaggcgccagcttcatccagatgtctgttcccaggacaagaatacttctggtcatgaactttttg

SEQ ID NO: 8 - DNA, 201 bp, Oryza sativa
tcacatgatctgcaactgtcaacagtcttaccggaattggattctgaaggtggatactccacctgtccaccataagtccttatttgtcagaggttacaatygcatgatgtgtctatactctatactgcaaagatgaatactaacaagtttttcttgggcttaaaagaagaaaaactaggaacagcctcactagtttgctag

SEQ ID NO: 9 - DNA, 201 bp, Oryza sativa
tgtttcaagtttggttgctgaaaaacgtacggacaaaccatgaactaacttgctattttgctccacatgggtttgtctcgaagcaaccaggaattgatcarcttcggtggtttgccaagaacatgaaacctggggataaggatttttttcgactttgctaatgctggtcgtctggattaggaacagaacaggtattgctac

SEQ ID NO: 10 - DNA, 201 bp, Oryza sativa
agtctaaatgggctgcactttgattgggctgggttcatatgagattaggggaaaaaacacgaacattccagtaaaatggggagtgtgaactgtgaagaagrgggtaaacggtgtgcggacgtgagacgagaaaagcatgagagaaaacgatctgtgtgcatgcatagggctggacgaaaagctcgtgactcgttagctcgc

SEQ ID NO: 11 - DNA, 201 bp, Oryza sativa
tagggcttctgatagccctccatctgtccgtcctttgcccgtttgcttcttggcctaaaccaccgaaaaggtgggtccgttttgctggacgcctggaataytcttcaactcgattggaacagcaggctccgtgtatgtgtaactatggctgtgtttagatctaaagtttagattcaaagtatagatttaaacttcagtcat

SEQ ID NO: 12 - DNA, 201 bp, Oryza sativa
tgctgattctcaggctgattctacttggttggtagaaaatctacttatccaggaacaagcgtagggtaacttttcctttttttctcagctatgtgaaaagrgagaaaactcgctacactttataggaaatgaactactcttctaccgacggatatcctaaaggctatcctctggtacctcggccttacgctaactcaaaac

SEQ ID NO: 13 - DNA, 201 bp, Oryza sativa
cgatcccagggaggttgtggaagtgcttctcatgaccttcgaggcactgcggcgtaggcatcttcaattggatgagacacaagagactagcaaacgtgcaracctgaaggctggtgccatcatgttggccagtaatctgagggctaacattgggaagaggattggagctgtccctggagttgaagtaggggatattttcta

SEQ ID NO: 14 - DNA, 201 bp, Oryza sativa
aattccaatttcatcccatttgtcccattccctcctgattactttgccaagaaaaataagcctgtggagaattcatcagatgcaggaatagtgccagaagrccctccatcagctgaaaaattaccagaaacaaaatattcatctggaaatctgggaaattttcagaacagctcacaggtgatgggcagtcaggcagcaaac

SEQ ID NO: 15 - DNA, 201 bp, Oryza sativa
gttttggttgctattaatcgattgagcaagtaggggaaatattcctatcatctatgcttcaaataaagttttctcttaaattactcatccgatttacaatycgattacaccgttgtgttcgtaataattaaatctttacaacaagatctcacatgattatattttgatgaaaaatcacaaattacttttatgatatgtcta

SEQ ID NO: 16 - DNA, 201 bp, Oryza sativa
gtcccgcctggtgacgatttccatgggcattgcgccgactgactgtgtcggcagcatgcatcgtctcgggcgttcaacgtgtggaggggacgacgtataaragtacacgcgaagactgtaggtagaggtgcttttcccgcgaaaagtggcagtagcggcggttggacagtaaccttcgtgtatggttgtgtgttcatctca

SEQ ID NO: 17 - DNA, 201 bp, Oryza sativa
tgcttgtgcgttcactgttcagagaagctggttatcctccctgataagaacagccgggaggtcagtgtgctatggttttgtttagttctggaatgatccartcacccagcacaattgactggctgagtgttgcattaagcaaatctggaccggatttgagggaattttctcgcgcagtggagatctatgataaatctcgta

SEQ ID NO: 18 - DNA, 201 bp, Oryza sativa
ctgcttcgccaacggcctcgaggcgaggctggcaggtactggtagtcaaatttacaagaactacacgataactcggcttccatgcactgatgtgctgaaarcgtaccagctttatttggcagcttgcccatttaagaagatctctcattactttgccaatcaaacaattttgaatgctgtggagaaggccaagaaagttca

SEQ ID NO: 19 - DNA, 201 bp, Oryza sativa
tcacattctggttgttgagggtccactgatacctttacctgttgcagtttattgttttaaataatccaatcaaacttttgtttgagcttattgctgaatarcacagcagcagtacatgcaatgcaagatgcccagatgatgagaataaaggcaatggcaaaaatataagtgctagttctatttcaaaataacaaacagaca

SEQ ID NO: 20 - DNA, 201 bp, Oryza sativa
tatgatgatgcttattatagcctaaggtatgtacttttaagatttagttcgaagtaatgcccatctggcaagttaattccagcattaacgtgttctaaaarccactctacttatgagaagccgggccaccacattcatacattacagccagaaacaacaaatccaggaagttaatacgtgattaagaatgcatcaaacaag

SEQ ID NO: 21 - DNA, 201 bp, Oryza sativa
tcgatatgttgggttttttctctttactagtagcatgccatctagtgtgcatcttacgtagtggaatattatcgggcacccaatattcggctcgcacaaarctccgaggacgaggaggaggacgactaatttggcagctcagctcacctgcacggctgcactgtgctgtgcccggtgggcgaagccatttcacccgcgggc

SEQ ID NO: 22 - DNA, 201 bp, Oryza sativa
tctgaaaacgcatggccgaaataagatgcaagaacacctgcaaaataatctcaggatcagtccaggtacgcattctctactgttatctactgaaccagagrggaaaaaaacaaaaactaggatgaatgcagtgtcactttgctgcttgtaattctctgaatttctgaatgaaagaaaagaaaagaaaagaagcgaaactgg

SEQ ID NO: 23 - DNA, 201 bp, Oryza sativa
cttaaattctcatgttttattcccgttgcaacgaacggtcatttcttttagtgtccataaatagctataagaggcatcgatcatcgcagcaagccgactgrgtgtggcgcctacgtgatcgttggtttgtttcgcttgtttgggcatacagctatgagaactttgttgggggcccatactacttatcatcatgtgtctaat

SEQ ID NO: 24 - DNA, 201 bp, Oryza sativa
gaactaaacacacccggaatgtgatggatccgaatctgctgtagttgatactgtgaatgtaacttgtaggcctcatttgattttctagaaaaaaatggagraaaaacataggaataagaatcctatgtgaattggtactgttcatccctttgatttgtaggaattgaacaaaggaaaagcatggggaaaaaaatcctatga

SEQ ID NO: 25 - DNA, 201 bp, Oryza sativa
agcgccacgccgcggccagcgccgtggtgttctccgggtggcatcgcttgagctacatcaccaccgatggccacttaaagtccgttgagctcgatcgccaratccggcggctccacagggccgtcggcaacgcggtcgtcgacgacaagtacttggtcttcgggaccggctccacccacctgatcaacgcgctggtgtacg

SEQ ID NO: 26 - DNA, 201 bp, Oryza sativa
acgggcggtaccagctacctgtcacagacatgtgggcccagcttaacgctaacgcgctgatggccccacatggcagcgacctgccccctctgtccctccgytccacgggcgcaccgagcgtccaccgccccccgcgatatccgggggtttaggcgatatttagccacgagagggggaggggagagtaggagaccgacgctt

SEQ ID NO: 27 - DNA, 201 bp, Oryza sativa
agaaagacttgctttagctttattgtttcttttccatattctatattcttgaaaaggactgcaaagctcttctagtatatgcaattagctgctttggaagrcacttcaaaagggatgaaggaaagaaggctgtcatatcaattactcaatcatgaccagatcatcgatctgatgcagttaaaaatttcattaattttgcca

SEQ ID NO: 28 - DNA, 401 bp, Oryza sativa
atcgatgtaattagtgatgtcaatcaatggtccagatggcatttggagtcttcgagccttatctttagtgtcacttgcattttcagttccaaatgaacatctggaagaaggcttggatatctttggaatttcattgataggatgaaaatctcttgccgcatgaagcctgacggagtttccgttagccaaagtggcatcagrtacagcatattccaaggaatctgtgtgcttcctatcaggttttgctggaatggaaaattgtgctggctcagttttgctgttccccctacttttcaataaatcaggttcaccttcttttcgcagaccagttgaattttgtatattctctttacaagcagatgctgaagagtggcctaataaattatttggtgaaacctcta

SEQ ID NO: 29 - DNA, 401 bp, Oryza sativa
taaccttatagtgggacaaggactgaaaagcagttcctcttgctttaacccagagagggtcaacatttttctccctgtaagttccaatgctccacaatatttgtatcaagtgttttgaggttccaggatatgcttcagaatccattgctccccatctcaatagaatgcataagctgaaaaggcaagaaaaagtggaataaraaatagattttctacaagcacatgatcattggtgggcactgcccacagataaaactagctagctctcggcagtcttacccatgggaaacagtaggatctatcgaaaaatcaagcagctgctttgatataactttccaggcagtatagaaatctggcaaagagattagcagctcacctcagaagtgaaatttggagggcaa

SEQ ID NO: 30 - DNA, 398 bp, Oryza sativa
ccaagcggagacatcgcttccatgagcaattcacggtttttcactagatctctcaccctttctctgatccattctggaccagcctctaatgcgtagagcgccaggcgctgcccgatgatggaagcacagataggtatgttatcttgcactttgagcagctgtgcatgaagaccgtcagcttcgtttgggtgggcaatmtgcagcagtcagctcatcagttcttgtaagactcactgatcaacacagattgtgcagccactaagttacttatactgcattgctatggtgataatttaagggaatgccctggtaaaagattcaagtggatgcgggaaattcatgaaactgaaagaactcaatattgactcttacatcagcattttcaagcctaagcagag

SEQ ID NO: 31 - DNA, 401 bp, Oryza sativa
tttaaatcaaatcttaaaaatataaatcataaataactatcaagttgttgagtttaaaaatataaaaattatataaatatatttgtcttgaaaaatactttcataaaagtatacatatatcactttttaataaatatttttataaaaacaagaagtcaaagttatgttttagagaccgcgtctctgttctaaacgacttcytttataagtatggagggagtatccatttcacatatacttatggtcttgtttacatcccaacaaattttagccaaaaacatcacatcaaatatttagccacatgtataggacattaaatataaaaaaacaattacacagtttgcatgtaaattgcgagacgaatcttttgagcctaattacgccattatttgacaatgtgg

SEQ ID NO: 32 - DNA, 401 bp, Oryza sativa
cggaactatgactaactcctctccgtaagcttctttgtaatatgtattgctgctgtacttggtctcattatctccttacagatatatatacattttttgcagggtatatccacttcatcttctccgtgacattgagactagggtttggctcctggccgtggagtcagagagtcagtgtaaagctgacggagaatatgcacyttccagtgttactcaaaatctagctactggaaacaataccaatattatagaacaaacagctgatgttatcacaaaaatagacaatagtatgagttcaccacggatgagaataacagaaaggaatggtataagggacaacaccaccccatcattccatcaacatttgcaactctttgagtctaatggcgaaggcgtacata

SEQ ID NO: 33 - DNA, 375 bp, Oryza sativa
caactactgacaacaagtgccatgtctaaatttctgaacatgcacacaacacacaaatgatgaatatggtgaaaccgcaattagcattagaaagttttaactctagaaatcaatttccaagttgtaatccccatactcccaacccagaagggaaaaaaaacaactccaaaacccycaacttttaaaaatgtgggaacaatcaaaccatatgcttgagatatacccacaaagccatcggcggccgcttacagcagagtacaccctcatcttgcacgcctccgaagaagcaggagccgtgatcaacacgagcatcttgtcctgctccaccccacacagtgacgagtctagggcacgacgaaggcgcgctcctaaacc

SEQ ID NO: 34 - DNA, 401 bp, Oryza sativa
cttcctgtcgtgagtgactgggtggtgggctcaatcggcctggcccgatacgatgcaagcgcgtggctgggcaggagatcggacggtgctgattgttggggcgacgtggccgcgtgggcgaatgaatagtgaacagtaccgacgtgaggtttataggattttatatgactaggggtgaacgttggatagaagggaatgtgytagtgctgttctgaacctcttgcgcatacattaacatgttttatctaatctaataaacatgattaaatttagcgtttgcttttacagtagtagaaatatgaaattgaacaatggttagtctgaggaatcataagcctatgatctagctggagtcttctccggtttaagctaccaattgaaacatattaattgatgcctga

SEQ ID NO: 35 - DNA, 401 bp, Oryza sativa
aatgtgctcaacttcatatatatgtgtgttgagcacatagctcatatataagatcaatggttagatcaatggtttttgggttagatcaatggttgagcacatagctcatatatatgtgtgctcaacggctcacacacaacttcatatatatgtacccaaaaaagcactattagatcaatggttataattgtttcaccacgraatattcaactttactcaatgttttgtttaacaagttccttttggtcacttgccaatttttctagatcatacagtacaatctattgatcacaattcacattgaataactaggtcaagccattctgtacatgcccatgcatgaacttactgtactaatattatcttagattaatttatcctgaaacttatagtcatatgtg

SEQ ID NO: 36 - DNA, 201 bp, Oryza sativa
  misc_feature (102)..(102): May or may not be present
gcatgaaagctgagaccatcaccaggttgatcgttgttgctgctattataagatgccaaaatcggcaaatcggtcattcactcaaggattggacacaagacaaaaaaaaagtaacaggtagcagactttcaactaacctggcatgaaagcttggattgtcactggtttgattgttgctgctgctgttatgaaagctgtata

SEQ ID NO: 37 - DNA, 201 bp, Oryza sativa
acgttgcttaggtagcaccttgatttaatcaaatgctagctagttgatgccaggtggcacactgcggacggatttgtttgtcagtttccctgcattacacwttgtacaggagtgtactacatccacatacaatgaacagtagtagtagcagcagctatatactccagttgcctagtcgtacacaaagtataattaatcaca

SEQ ID NO: 38 - DNA, 401 bp, Oryza sativa
gccggcgcagcgagaagagtgccgaatgttggatggaggacgccgaagcgcgggaaggtcatggtggcggcgttctggctccgtccacgtcggactagcgacgcgtggtcgacgacccctgtgctgcatcctaccatgccaactttgcgtatccgtcggcgtccatcttcgccaggatgccggggaaggagaagaagaggcggcggcgaggccgaagaggcgaggatagggatgaggtggcggaggaggggcgtgggaggggaggcagcgagctcccgccgccccgtcactcctgccgctctcgtcgccccgccattccgccgagcttccgccgccctgtcgttcccgccgccccgccattccgccactccgccgagctcccgccgccccgcctctcccgc

SEQ ID NO: 39 - DNA, 401 bp, Oryza sativa
acgcgcgcgcctccattgttctcggatcaacaagctctccaagaacagcagcaaagatgaagccttcgtcttcctccgtcggcgtctgtaccctgctggtggcggtggcctccctgcagctcctcctcgtcgtcgccgtcgccgcctcggcgaagactgcaccggcgatgccagacgaggagttcttgggccgtctctgcgaccagcagcagggggccacgcggcggcggctcccgtggtgccagcagctgcacgcgaggcggcgccacggcggtggcggcggcggcgtcggcgtcggcaagcggcggcgggtgccgatgccgccgcccagccgcgccggcgaggagatcgacgcgcgctacgacgtgtccaagcgggtcgtgccgagcggaccgaacccg

SEQ ID NO: 40 - DNA, 401 bp, Oryza sativa
ttttggggtcttcccttcttattttccctgagcgtagaaaattctgtggtttccagttttccacggaagtaaattccaattttccaatagatgtacgtcaaccctttgcttcctctccagctgcagagttgcaggtttgacgaatgcagcttatctacaaaattcccatcagagggaacacagttacagaagaactaggggaagtacagattgcaaatccataaggatcttctttagaaccgtatacgtaaagggcttcatggattggccactatatatgggtgtcaccctcaatcgtgaatctgcaaggtcagatatcagtatatcaaatgcagattgcctcattgcagattgctgtggattgttcaggttccgggttagcccagtcaccagtcttcact

SEQ ID NO: 41 - DNA, 401 bp, Oryza sativa
ccacgcgagcagctggtgtttgctcatggtggcagtggtgcgcgataccagtagcgtgcgcgacgcgtcggggtggtcatcggcgagggcgagcatgtcgtcgtccagtggacgcggactctagggtgatcacgctcggccctgtcacgctcaaaacaatactacggcacatctgattacgttgacaggatctgagaccacaccagaactatcccattccgatcatgcatgtgaaaaaaaaaacaaaggccaactattccatttagcagtaatcaagatccgatcttctcttttcttgtgaaaattcgacatgtttccggttaccaaccgaggaacacagattaattactctagttttttcgaagagcagaagaggaatattgattacccccacaaaaccc

SEQ ID NO: 42 - DNA, 401 bp, Oryza sativa
caacactctaaaagttttttttttacccgttcacttgccttgttagtctatctgtactttatgatcataaatagttttataataaagcatgacggatttttgtttcaagtttggttgctgaaaaacgtacggacaaaccatgaactaacttgctattttgctccacatgggtttgtctcgaagcaaccaggaattgatcaacttcggtggtttgccaagaacatgaaacctggggataaggatttttttcgactttgctaatgctggtcgtctggattaggaacagaacaggtattgctactgcttttattcctaagcttctaatacttctgctcatacggatacggccatatacatacataggagtagattcgatttgacgtctcaagcagtagatgctg

SEQ ID NO: 43 - DNA, 401 bp, Oryza sativa
ggtaggcacggcccgacgaggcccatcgggagccgccgccgcgtgcccacgcctcatatataaaggccaccgcgtcctctcgcctccgccagtccgcctccctcacaaccctaaccctaaccctagccgcctccgccgatccacgcacgcctccgcctccgcctccgccttgaccgctccgcctccgcttccgcctccgtcgatccacgcctccacctccacgcgaccacgcctccatctctccatccctctccgtcgccgtctctgatgaacgccttgccggatctaccaccgagggtcgctgcctcgccggatccgtgaccttgtctcatctccgcctctccagtctttggatcgttggccgtgctctcgatttcctctttctttttcattttttttgc

SEQ ID NO: 44 - DNA, 401 bp, Oryza sativa
ttcacggattgctcctcacgcgcaatggaatggcagcagcctcctcggccgtcgcccacgtgtcacgagtgcgctcaggcagctgggccttgattccttgagtctaaatgggctgcactttgattgggctgggttcatatgagattaggggaaaaaacacgaacattccagtaaaatggggagtgtgaactgtgaagaagggggtaaacggtgtgcggacgtgagacgagaaaagcatgagagaaaacgatctgtgtgcatgcatagggctggacgaaaagctcgtgactcgttagctcgctcggttcgtgtctggctcggctcggctcggctcggctcgtttggatttgttaacgagccgagctaaggtttcagctcgttatctataacgagccagctcg

SEQ ID NO: 45 - DNA, 401 bp, Oryza sativa
gaaccgaatgacttgttgtatacgttgctcctgcttctctgcctgatccctctctgatgatggtgtgtgtcccttttgtttcgcttttcttaatcctctctagggcttctgatagccctccatctgtccgtcctttgcccgtttgcttcttggcctaaaccaccgaaaaggtgggtccgttttgctggacgcctggaatactcttcaactcgattggaacagcaggctccgtgtatgtgtaactatggctgtgtttagatctaaagtttagattcaaagtatagatttaaacttcagtcatttttcatcacatcaacctgtcatatacacacaactttttagtcacatcatctttaattttaaccaaaatataaattttacgctgaactaaacacagtata

SEQ ID NO: 46 - DNA, 401 bp, Oryza sativa
ccctcgacctcgtcggtgggaggaggacgacggcggtggggaagaacctgaggcggcagcgagagagacaggcggtgtcgccggagcagtgaggagggaggcggcgtcgagagagagaagagagaggcgatggcgacgacgaccggatccgcgacggcgacgacggatccgcggcgacgacaaccggatccggtggcctcctccacctccgccttggcctcctcgacctcggccaccgcgacctcctccacctccgtcttggcctcctctgcgtggcggcgagagagaggcaagcagcagcggcgagagagagagaggagaaagcggcggcggcggtggctggggaggtggcgccggcgctcgcgggagagagagggagagggaggggaggacggcgacgg

SEQ ID NO: 47 - DNA, 401 bp, Oryza sativa
cggcagcgagagagacaggcggtgtcgccggagcagtgaggagggaggcggcgtcgagagagagaagagagaggcgatggcgacgacgaccggatccgcgacggcgacgacggatccgcggcgacgacaaccggatccggtggcctcctccacctccgccttggcctcctcgacctcggccaccgcgacctcctccacctccgtcttggcctcctctgcgtggcggcgagagagaggcaagcagcagcggcgagagagagagaggagaaagcggcggcggcggtggctggggaggtggcgccggcgctcgcgggagagagagggagagggaggggaggacggcgacggcaccgagtggagggagtgaggtggcgtggagcgaagaaaaaagaagaggaggg

SEQ ID NO: 48 - DNA, 401 bp, Oryza sativa
aagacccgcagtgcgaggatttcgaggatcaagctccagatctcgagcaaggcaagccacctttgaacatcttgagcctatatttgaaatttaattatgttgcttgaaaaatattatgcattgataggatcgcacttaatctgtcgtcccgtctgcaaggcagattggcggacccacctaatttgttgcattgatcctcccttgttaattgttatatcatgtccccctgtaaccatctagttgcgtctcgacattcgcgcaccctgtgcgagcatcgacggacgccttcaaacttaaaatctgaaaaacaacttgggtaaaacttgggtttacaaaagacttggaaaactcgacacctgggtcggtgcttgcgaactaaatggattttccaaaaccgcgga

SEQ ID NO: 49 - DNA, 401 bp, Oryza sativa
gaacacccacacaatctcgatttgattgagaatctaggaggatactgattggcgctcaagaatggcgtagttaatgttatgatttgccagcattctcagctgctgattctcaggctgattctacttggttggtagaaaatctacttatccaggaacaagcgtagggtaacttttcctttttttctcagctatgtgaaaagggagaaaactcgctacactttataggaaatgaactactcttctaccgacggatatcctaaaggctatcctctggtacctcggccttacgctaactcaaaaccaaactaaaatgggttgatcggagctattctctagaatttttgacccaaattgagcgaaggcggccacttcgcgatattgtgccaattccagtgctcgaa

SEQ ID NO: 50 - DNA, 401 bp, Oryza sativa
tagcagcagatgtcatacaaacaggctttcattggaagcaataaaaatagtggacatccaaaagatgtgtggaactatgacttctagatatcacaggcatctagcatcttgatttttattcaagactgcacataacatctttacattctagagggaaatgatccgacttaagtagtttgatagttcacctcagggaggaagtcctttgatagtgttatagatgtctcccgaagcaccttgactgccacttcctctccattgtccaatatgccatgataaaccataccaaatcctccttttccaatgatagactggaagttgttagttatagtcttcaactctgtatatgtgaatcttctggtgtcagtatgcaggggagtatcctcttcatacatatcata

SEQ ID NO: 51 - DNA, 401 bp, Oryza sativa
gtttgggcaccgacagctccaacggaacaaagaaacgccctaagacctctaataggaaggctgctactgacaatgagatttccttgatgcctccatccagcgatcccagggaggttgtggaagtgcttctcatgaccttcgaggcactgcggcgtaggcatcttcaattggatgagacacaagagactagcaaacgtgcagacctgaaggctggtgccatcatgttggccagtaatctgagggctaacattgggaagaggattggagctgtccctggagttgaagtaggggatattttctacttcaggatggagctatgcattatcggcttgcatgcacctagcatgggtggaattgattatatgaataagtttggtgatgaggatgactctgtagcaata

SEQ ID NO: 52 - DNA, 401 bp, Oryza sativa
aatgaggaaaggtgagaatcggtttgttattagtaagaagaaagaccgctcactgacatcgccacagtacaaaaggcgcagtgtgctcgagcatgctgataattccaatttcatcccatttgtcccattccctcctgattactttgccaagaaaaataagcctgtggagaattcatcagatgcaggaatagtgccagaaggccctccatcagctgaaaaattaccagaaacaaaatattcatctggaaatctgggaaattttcagaacagctcacaggtgatgggcagtcaggcagcaaacaacatgaacaatgagaacaggaacggaaattatccacatcaaaacttgagtacaagtggttatgggtatggtgaaagcatcacttatcagcatcaaccac

SEQ ID NO: 53 - DNA, 401 bp, Oryza sativa
tgatttggttgatttgtgggcgcgcgcgcgcatggcgaaggtacatcctaacgtggtgcccgtggcggcggcggcagggccggccggcggcgagcggcggggggaggaggaggaggaggcggcggcgctgacggtgtggcggaagtcgctgctgttcaactgcaaggggttcacggtgttcgacgccaaggggaacctggcgtaccgcgtcgacagctacgacacggagagcggcgacgaggtcgtcctcatggacgccgccggcgccccggccttcaccgtccgcaggaagaggcagctcagcctgcagggggagcagtggctcgtgttcgccggcgaggcggacggccggcggccgcccgtgtacgcggtcaggcggacgggccgcggcggcggcaagt

SEQ ID NO: 54 - DNA, 401 bp, Oryza sativa
aaaaaatatggtttcaaagttttccaaatcggtaaatctaattggagaggcctctccaattagtcttaaccagagacacccacgtgctagtactttaggagttttggttgctattaatcgattgagcaagtaggggaaatattcctatcatctatgcttcaaataaagttttctcttaaattactcatccgatttacaatccgattacaccgttgtgttcgtaataattaaatctttacaacaagatctcacatgattatattttgatgaaaaatcacaaattacttttatgatatgtctaaattacttttagatttcactaagttacttcttagacatataaaagtaaattcagtaaagcctaaaagtaattacatatattatagcagtaacttataaca

SEQ ID NO: 55 - DNA, 401 bp, Oryza sativa
aacgtcgacgagaaccgggctcccaactgacggtcacgcgagagctgcacgaaacgagcctcgacgacgatcccatccgtccgtccgtcgctgcggctgctgctgctgccgccacaggcggtcagagcctctggcacgatgccaacacgcgggcacgtggtagggcagcacgggccattcaggtggtgtttggatccagggacttaactttattctctatatttagacactaatttaaaatattaaatatagattacttacaaaactaattacataaatgaaagctaatttgtgtgataacttttttaagcttaattaatccataattagagaatgtttaatgtagcatcacataagctaatcatggattaattaggctcaatagattcgtctcgcgaatt

SEQ ID NO: 56 - DNA, 401 bp, Oryza sativa
cgtccgccgaagcgcacgaccggcgcggcgtggggagcggcgagtcgagcagctgcgggagcttctcgccgtcggcgccattgcaccgcagcccctccttgtcccgcctggtgacgatttccatgggcattgcgccgactgactgtgtcggcagcatgcatcgtctcgggcgttcaacgtgtggaggggacgacgtataagagtacacgcgaagactgtaggtagaggtgcttttcccgcgaaaagtggcagtagcggcggttggacagtaaccttcgtgtatggttgtgtgttcatctcacgtactgttcttttgcctctcgctagctcgttcccgtgatcaaggtgcatgctcgatggccttaatggtggaggttgccgaaaggtagcagaggaaatca

SEQ ID NO: 57 - DNA, 401 bp, Oryza sativa
ggatggatagtaaatataatatgaattgatctattggatcagttatatatatatatatatatatatatatatatatatatatatatatatatatatagacacacacacacacaatgaggatggtaaattagtgacaatatatgaatgtgttctattgtcaaaacgaaagggatcgatgagttatatctctaggttaattagtttacaacgaagagttgaagctggaataaacaagtcaaaattatatctgtataacatcatagtaatgccgaccatgtacgcatccacatggccatacagcaacatcagaaacagaatttaattaattatttgactaaacccagaatcatttgctgctgcatcgaatcgttcctctcgtcatcgccgacgcaaacatgcgc

SEQ ID NO: 58 - DNA, 401 bp, Oryza sativa
ctatgagttagctagctaacgtgtatgatgtccaatgattaagtgacactttttttctgtctaatataatcatccatctcatcatatcattagctccttgtgcttgtgcgttcactgttcagagaagctggttatcctccctgataagaacagccgggaggtcagtgtgctatggttttgtttagttctggaatgatccagtcacccagcacaattgactggctgagtgttgcattaagcaaatctggaccggatttgagggaattttctcgcgcagtggagatctatgataaatctcgtaccgatccagcatagtgattcgtccgcgggattaatactgtaactaatccatagattagcgccattattgaaacacgctttcttcttattgttgttattat

SEQ ID NO: 59 - DNA, 401 bp, Oryza sativa
actctgtagtctgcaaggagcggtggcgagcagtggcgcgcgaagtcgatagggtggcgagcggacggagtggcgacggagagcctgcgggagtcgagatcgtccggggaagcaacgacggcaacgacggcagccttgtatcccgtcggcgaggtcacgctcggccattgcgcacctctcccttcgcccatcgccatcgagcccccacccacggcgcccggccatccccggcgaggagctctgtttttggtgggtgtcggcggagttggaacgaaggagggtcgttctcggcatcgatgtcgccatctccgatcctccaccgccaccgccgccctccccccctccattgccgacccctccccggcgtcgagaaaatcctcgcccgacctcagcaacaagaa

SEQ ID NO: 60 - DNA, 401 bp, Oryza sativa
tagactgcatcgccacctgccgccgaactgcgccgtgctgccgcccgccggtgccctctccttcacctcccgctgcatcgccgcctgccgccaagcgcacggcgaagggtaaggagtcgtggcggcgcggggcgctcatggcggtggaggacctgctggatgttgctgctcctgttctcgccattgtcggagtcggcgccgcccacgccgacggagaatctcaaggaggcgatgagcacgccgaggctcggacccagcttcgtcggtgggacaaagcgggactcgatggagacggtggagctctcctcctcctcccccaacaccacctcatgtagcttccccctcggcgcgtcagtaggtaggggtatccatcgcttgtgcagctgcaccgagtcctcatc

SEQ ID NO: 61 - DNA, 401 bp, Oryza sativa
tcctggaggatgagcgtgagcgtgcgcgcaagatagcgcacgagatcaagggattcggcagcttcaacctcagcagcgcgcatgcgtcggggtcggcggcggcagccctccgcgcgggggcgatggagcaccagtgctacggccggagcaactcgcggtacgagggcaggtggaggagggaggcctgcgtggacgacggcgacaaggagaacctgctggtggtgtcgatggccgaggcgaaggccgaggcggcggcggaggagccgcaccactaccaccacccgttctacggcttcgggcagcagcggccggaggcgatgctgctcctgagccagtagtgatcgtttgggtggatggttcttcgtcgatcgcatcgttcgttggtttgtgatgcgtgagaa

SEQ ID NO: 62 - DNA, 401 bp, Oryza sativa
agtctgtggccactgatgacaggcgcagtgcaactgagctcctgaagcagatcaggcagcatgctcatgccaatggtgatggtgatcagcgtttggcacactgcttcgccaacggcctcgaggcgaggctggcaggtactggtagtcaaatttacaagaactacacgataactcggcttccatgcactgatgtgctgaaagcgtaccagctttatttggcagcttgcccatttaagaagatctctcattactttgccaatcaaacaattttgaatgctgtggagaaggccaagaaagttcacattgtcgattatggcatatactatggatttcagtggccgtgtcttattcagcggctatctaacaggcctggaggcccaccaaagcttaggatcactgga

SEQ ID NO: 63 - DNA, 401 bp, Oryza sativa
gggcattggtgaaggctcagtaaccggaggtcttgtttgatggttggcaactgaattgttaattaccaatttatttcctgtgcttctaataccagcagcatcacattctggttgttgagggtccactgatacctttacctgttgcagtttattgttttaaataatccaatcaaacttttgtttgagcttattgctgaatagcacagcagcagtacatgcaatgcaagatgcccagatgatgagaataaaggcaatggcaaaaatataagtgctagttctatttcaaaataacaaacagacaacattgcattctaaacttttataaccaaacaaacaaaggaaacagggaaaattgctgaattaatgttccctttactaagtaaattctactagaaagcact

SEQ ID NO: 64 - DNA, 201 bp, Oryza sativa; identical to SEQ ID NO: 7

SEQ ID NO: 65 - DNA, 201 bp, Oryza sativa; identical to SEQ ID NO: 8